European Patent Application EP 4 218 787 A2, published August 2, 2023. Title: Peptides for treating muscle atrophy. Applicant: Nuritas Limited. Application EP. The sequence listing filed with the application follows.

SEQUENCE LISTING (20 sequences)

SEQ ID NO: 1 - protein, 8 aa, Vicia faba
TIKLPAGT

SEQ ID NO: 2 - protein, 9 aa, Vicia faba
IEDPGQFPT

SEQ ID NO: 3 - protein, 10 aa, Vicia faba
HLPSYSPSPQ

SEQ ID NO: 4 - protein, 13 aa, Vicia faba
KGDIIAIPSGIPY

SEQ ID NO: 5 - protein, 8 aa, Vicia faba
LDWYKGPT

SEQ ID NO: 6 - protein, 8 aa, Vicia faba
SRGPIYSN

SEQ ID NO: 7 - protein, 13 aa, Vicia faba
LERGDTIKIPAGT

SEQ ID NO: 8 - protein, 8 aa, Vicia faba
TIKIPAGT

SEQ ID NO: 9 - protein, 7 aa, Vicia faba
SYSPSPQ

SEQ ID NO: 10 - protein, 19 aa, Vicia faba
IGSSSSPDIYNPQAGRIKT

SEQ ID NO: 11 - protein, 17 aa, Vicia faba
IDPNGLHLPSYSPSPQL

SEQ ID NO: 12 - protein, 18 aa, Vicia faba
LVNRDDEEDLRVLDLVIP

SEQ ID NO: 13 - protein, 16 aa, Vicia faba
ITGQVLHPNGGTVVNA

SEQ ID NO: 14 - protein, 7 aa, Vicia faba
ALEPDNR

SEQ ID NO: 15 - protein, 14 aa, Vicia faba
LREQSQQNECQLER

SEQ ID NO: 16 - protein, 20 aa, Vicia faba
VAGKGIPWDKQDPGEEAIES

SEQ ID NO: 17 - protein, 19 aa, Vicia faba
VGRRGGQHQQEEESEEQKD

SEQ ID NO: 18 - protein, 14 aa, Vicia faba
YDEEKEQGEEEIRK

SEQ ID NO: 19 - protein, 9 aa, Vicia faba
HLPSYSPSP

SEQ ID NO: 20 - protein, 6 aa, Vicia faba
SYSPSP